European Patent Application EP 4 635 575 A1, published October 22, 2025. Title: Uniwersalne przeciwciało monoklonalne do eliminowania komórek opornych na działanie przeciwciał antynowotworowych pierwszego rzutu. Applicant: Gdański Uniwersytet Medyczny. Application PL. The sequence listing filed with the application follows.

SEQUENCE LISTING (2 sequences)

SEQ ID NO: 1 - protein, 452 aa, synthetic construct
QSVEESGGRLVTPGTPLTLTCTVSGFSLSSYAMGWFRQAPGKGLEWIGFINIGGRASYASWAKGRFTISKTSTTVDLKMTSPTTEDTATYFCARGRAYTLTGGTYTRAFDPWGPGTLVTVSSASTKGPSVFPLAPSSKSTSGGTAALGCLVKDYFPEPVTVSWNSGALTSGVHTFPAVLQSSGLYSLSSVVTVPSSSLGTQTYICNVNHKPSNTKVDKKVEPKSCDKTHTCPPCPAPELLGGPSVFLFPPKPKDTLMISRTPEVTCVVVDVSHEDPEVKFNWYVDGVEVHNAKTKPREEQYNSTYRVVSVLTVLHQDWLNGKEYKCKVSNKALPAPIEKTISKAKGQPRRPQVYTLPPSRDELTKNQVSLTCLVKGFYPSDIAVEWESNGQPENNYKTTPPVLDSDGSFFLYSKLTVDKSRWQQGNVFSCSVMHGALHNHYTQKSLSLSPGK

SEQ ID NO: 2 - protein, 217 aa, synthetic construct
AQVLTQTASPVSAAVGSTVTINCQSSQKVYGNNNLAWYRQKPGQPPKVLIYAASTLASGVPSRFKGYGSGTQFTLTISDLECDDAATYYCAGAYGGDIYPFGGGTELEIKRTVAAPSVFIFPPSDEQLKSGTASVVCLLNNFYPREAKVQWKVDNALQSGNSQESVTEQDSKDSTYSLSSTLTLSKADYEKHKVYACEVTHQGLSSPVTKSFNRGEC